European Patent Application EP 4 578 287 A1, published July 2, 2025. Title: COMPOSITION FOR IMPROVING PLANT DROUGHT STRESS RESISTANCE COMPRISING TRICHODERMA-MEDIATED IRON OXIDE NANOPARTICLES AND METHOD FOR PRODUCING TRICHODERMA-MEDIATED IRON OXIDE NANOPARTICLES. Applicant: Seoul National University R&DB Foundation. The sequence listing filed with the application follows.

SEQUENCE LISTING (2 sequences)

SEQ ID NO: 1 - RNA, 624 nt, trichoderma harzianum
  source 1..624: mol_type = genomic RNA
gaagtaaaagtcgtaacaaggtctccgttggtgaaccagcggagggatcattaccgagtttacaactcccaaacccaatgtgaacgttaccaaactgttgcctcggcgggatctctgccccgggtgcgtcgcagccccggaccaaggcgcccgccggaggaccaaccaaaactctttttgtataccccctcgcgggttttttataatctgagccttctcggcgcctctcgtaggcgtttcgaaaatgaatcaaaactttcaacaacggatctcttggttctggcatcgatgaagaacgcagcgaaatgcgataagtaatgtgaattgcagaattcagtgaatcatcgaatctttgaacgcacattgcgcccgccagtattctggcgggcatgcctgtccgagcgtcatttcaaccctcgaacccctccggggggtcggcgttggggatcggccctgccttttggcggtggccgtctccgaaatacagtggcggtctcgccgcagcctctcctgcgcagtagtttgcacactcgcatcgggagcgcggcgcgtccacagccgttaaacacccaacttctgaaatgttgacctcggatcaggtaggaatacccgctgaacttaagc

SEQ ID NO: 2 - RNA, 623 nt, Trichoderma harzianum
  source 1..623: mol_type = genomic RNA
gaagtaaaagtcgtaacaaggtctccgttggtgaaccagcggagggatcattaccgagtttacaactcccaaacccaatgtgaacgttaccaaactgttgcctcggcgggatctctgccccgggtgcgtcgcagccccggaccaaggcgcccgccggaggaccaaccaaaactctttttgtataccccctcgcgggttttttataatctgagccttctcggcgcctctcgtaggcgtttcgaaaatgaatcaaaactttcaacaacggatctcttggttctggcatcgatgaagaacgcagcgaaatgcgataagtaatgtgaattgcagaattcagtgaatcatcgaatctttgaacgcacattgcgcccgccagtattctggcgggcatgcctgtccgagcgtcatttcaaccctcgaacccctccggggggtcggcgttggggatcggccctgcctttggcggtggccgtctccgaaatacagtggcggtctcgccgcagcctctcctgcgcagtagtttgcacactcgcatcgggagcgcggcgcgtccacagccgttaaacacccaacttctgaaatgttgacctcggatcaggtaggaatacccgctgaacttaagc